European Patent Application EP 4 378 485 A2, published June 5, 2024. Title: INTERNALIZING BINDING MOLECULES TARGETING RECEPTORS INVOLVED IN CELL PROLIFERATION OR CELL DIFFERENTIATION. Applicant: LinXis BV. Application EP. The sequence listing filed with the application follows.

SEQUENCE LISTING (371 sequences)

SEQ ID NO: 1 - protein, 113 aa, Lama glama
EVQLVESGGGLAQAGGSLRLSCVASGNIDSANGMAWYRQAPGKQRELVAHITSGTSYYVASVEGRFTISRANAKDTWYLQMNSLKPEDTGVYYCFPIGLSAHWSQGTQVTVSS

SEQ ID NO: 2 - protein, 25 aa, Lama glama
EVQLVESGGGLAQAGGSLRLSCVAS

SEQ ID NO: 3 - protein, 8 aa, Lama glama
GNIDSANG

SEQ ID NO: 4 - protein, 17 aa, Lama glama
MAWYRQAPGKQRELVAH

SEQ ID NO: 5 - protein, 6 aa, Lama glama
ITSGTS

SEQ ID NO: 6 - protein, 38 aa, Lama glama
YYVASVEGRFTISRANAKDTWYLQMNSLKPEDTGVYYC

SEQ ID NO: 7 - protein, 11 aa, Lama glama
FPIGLSAHWSQ

SEQ ID NO: 8 - protein, 8 aa, Lama glama
GTQVTVSS

SEQ ID NO: 9 - protein, 117 aa, Lama glama
EVQLVESGGGLVQAGGSLRLSCAASESISSIEQMGWFRQAPGKQRALVAINTYGGRTVYTNSVEGRFTMSRDSAKNMVYLQMTSLEPEDTAVYYCYAQTTAWRGGVWGQGTQVTVSS

SEQ ID NO: 10 - protein, 25 aa, Lama glama
EVQLVESGGGLVQAGGSLRLSCAAS

SEQ ID NO: 11 - protein, 8 aa, Lama glama
ESISSIEQ

SEQ ID NO: 12 - protein, 17 aa, Lama glama
MGWFRQAPGKQRALVAI

SEQ ID NO: 13 - protein, 7 aa, Lama glama
NTYGGRT

SEQ ID NO: 14 - protein, 38 aa, Lama glama
VYTNSVEGRFTMSRDSAKNMVYLQMTSLEPEDTAVYYC

SEQ ID NO: 15 - protein, 11 aa, Lama glama
YAQTTAWRGGV

SEQ ID NO: 16 - protein, 11 aa, Lama glama
WGQGTQVTVSS

SEQ ID NO: 17 - protein, 118 aa, Lama glama
EVQLVESGGGLVQAGGSARLSCAASGSILSPNLMAWSRQAPGKQREVVALATSDGITTYATSVKGRFTISRDDAKNTVYLQMNSLKPEDTNLYTCKYRALRAGAVDYWGQGTQVTVSS

SEQ ID NO: 18 - protein, 25 aa, Lama glama
EVQLVESGGGLVQAGGSARLSCAAS

SEQ ID NO: 19 - protein, 8 aa, Lama glama
GSILSPNL

SEQ ID NO: 20 - protein, 17 aa, Lama glama
MAWSRQAPGKQREVVAL

SEQ ID NO: 21 - protein, 7 aa, Lama glama
ATSDGIT

SEQ ID NO: 22 - protein, 38 aa, Lama glama
TYATSVKGRFTISRDDAKNTVYLQMNSLKPEDTNLYTC

SEQ ID NO: 23 - protein, 12 aa, Lama glama
KYRALRAGAVDY

SEQ ID NO: 24 - protein, 11 aa, Lama glama
WGQGTQVTVSS

SEQ ID NO: 25 - protein, 125 aa, Lama glama
EVQLVESGGGLVQAGGSLRLSCAASGRTSFSGYAMAWFRQAPGKERDFVASITWSYGYTYYTDSAQGRFTISRDSAKNTVYLEMNSLKPEDTAVYYCAADPKASRFRILREYAYWGQGTQVTVSS

SEQ ID NO: 26 - protein, 25 aa, Lama glama
EVQLVESGGGLVQAGGSLRLSCAAS

SEQ ID NO: 27 - protein, 9 aa, Lama glama
GRTSFSGYA

SEQ ID NO: 28 - protein, 17 aa, Lama glama
MAWFRQAPGKERDFVAS

SEQ ID NO: 29 - protein, 8 aa, Lama glama
ITWSYGYT

SEQ ID NO: 30 - protein, 38 aa, Lama glama
YYTDSAQGRFTISRDSAKNTVYLEMNSLKPEDTAVYYC

SEQ ID NO: 31 - protein, 17 aa, Lama glama
AADPKASRFRILREYAY

SEQ ID NO: 32 - protein, 11 aa, Lama glama
WGQGTQVTVSS

SEQ ID NO: 33 - protein, 129 aa, Lama glama
EVQLVESGGGSVQTGGSLRLSCAASGRSFSTYAMAWFRQAPGKEREFVAAINRRATDTVYADSAKGRFIISRDNDKNTVYLQMDSLKTEDTAVYYCAAAKNAYDWRWDRLRDRDYWGQRGQGTQVTVSS

SEQ ID NO: 34 - protein, 25 aa, Lama glama
EVQLVESGGGSVQTGGSLRLSCAAS

SEQ ID NO: 35 - protein, 8 aa, Lama glama
GRSFSTYA

SEQ ID NO: 36 - protein, 17 aa, Lama glama
MAWFRQAPGKEREFVAA

SEQ ID NO: 37 - protein, 8 aa, Lama glama
INRRATDT

SEQ ID NO: 38 - protein, 38 aa, Lama glama
VYADSAKGRFIISRDNDKNTVYLQMDSLKTEDTAVYYC

SEQ ID NO: 39 - protein, 19 aa, Lama glama
AAAKNAYDWRWDRLRDRDY

SEQ ID NO: 40 - protein, 14 aa, Lama glama
WGQRGQGTQVTVSS

SEQ ID NO: 41 - protein, 124 aa, Lama glama
EVQLVESGGGLVQAGGSLRLSCAASGRTFNGYAMAWFRQAPGKERDFVASITWSYGYTYYADSAQGRFTISRDSAKNTVYLEMNSLKPEDTAVYYCAADPKASRFRILRQYAHWGQGTQVTVSS

SEQ ID NO: 42 - protein, 25 aa, Lama glama
EVQLVESGGGLVQAGGSLRLSCAAS

SEQ ID NO: 43 - protein, 8 aa, Lama glama
GRTFNGYA

SEQ ID NO: 44 - protein, 17 aa, Lama glama
MAWFRQAPGKERDFVAS

SEQ ID NO: 45 - protein, 8 aa, Lama glama
ITWSYGYT

SEQ ID NO: 46 - protein, 38 aa, Lama glama
YYADSAQGRFTISRDSAKNTVYLEMNSLKPEDTAVYYC

SEQ ID NO: 47 - protein, 17 aa, Lama glama
AADPKASRFRILRQYAH

SEQ ID NO: 48 - protein, 11 aa, Lama glama
WGQGTQVTVSS

SEQ ID NO: 49 - protein, 124 aa, Lama glama
EVQLVESGGGLVQAGGSLRLSCAASGRTFNGYAMGWFRQAPGKERDFVAAITWSYGYTHYAESVKGRFSISRDSANNMVYLEMNSLKPEDTAVYYCAADPKASRFRTLRRYDYWGQGTQVTVSS

SEQ ID NO: 50 - protein, 25 aa, Lama glama
EVQLVESGGGLVQAGGSLRLSCAAS

SEQ ID NO: 51 - protein, 8 aa, Lama glama
GRTFNGYA

SEQ ID NO: 52 - protein, 17 aa, Lama glama
MGWFRQAPGKERDFVAA

SEQ ID NO: 53 - protein, 8 aa, Lama glama
ITWSYGYT

SEQ ID NO: 54 - protein, 38 aa, Lama glama
HYAESVKGRFSISRDSANNMVYLEMNSLKPEDTAVYYC

SEQ ID NO: 55 - protein, 17 aa, Lama glama
AADPKASRFRTLRRYDY

SEQ ID NO: 56 - protein, 11 aa, Lama glama
WGQGTQVTVSS

SEQ ID NO: 57 - protein, 127 aa, Lama glama
EVQLVESGGGLVQAGDSLRLSCAASGRTFSSYPIAWFRQAPGKEREFVAAITSSGLTTYYANVVKGRFAISRDNAKDTVYLQMNSLKPEDTAVHYCATSNGFLSGRDIYQHNKYIYWGQGTQVTVSS

SEQ ID NO: 58 - protein, 25 aa, Lama glama
EVQLVESGGGLVQAGDSLRLSCAAS

SEQ ID NO: 59 - protein, 8 aa, Lama glama
GRTFSSYP

SEQ ID NO: 60 - protein, 17 aa, Lama glama
IAWFRQAPGKEREFVAA

SEQ ID NO: 61 - protein, 5 aa, Lama glama
ITSSG

SEQ ID NO: 62 - protein, 41 aa, Lama glama
LTTYYANVVKGRFAISRDNAKDTVYLQMNSLKPEDTAVHYC

SEQ ID NO: 63 - protein, 20 aa, Lama glama
ATSNGFLSGRDIYQHNKYIY

SEQ ID NO: 64 - protein, 11 aa, Lama glama
WGQGTQVTVSS

SEQ ID NO: 65 - protein, 125 aa, Lama glama
EVQLVESGGGLVQAGGSLRLSCVISGRTSPTYPMGWFRQSPGNEREFVASINWSGGWRNYADSVKGRFTISRDDAKNTVYLQMNSLKPEDTAVYYCARGQYSSGTPVYAHEYAYWGQGTQVTVSS

SEQ ID NO: 66 - protein, 25 aa, Lama glama
EVQLVESGGGLVQAGGSLRLSCVIS

SEQ ID NO: 67 - protein, 8 aa, Lama glama
GRTSPTYP

SEQ ID NO: 68 - protein, 17 aa, Lama glama
MGWFRQSPGNEREFVAS

SEQ ID NO: 69 - protein, 8 aa, Lama glama
INWSGGWR

SEQ ID NO: 70 - protein, 38 aa, Lama glama
NYADSVKGRFTISRDDAKNTVYLQMNSLKPEDTAVYYC

SEQ ID NO: 71 - protein, 18 aa, Lama glama
ARGQYSSGTPVYAHEYAY

SEQ ID NO: 72 - protein, 11 aa, Lama glama
WGQGTQVTVSS

SEQ ID NO: 73 - protein, 117 aa, Lama glama
EVQLVESGGGLVQPGGSLRLSCAASESIFSINYMAWYRQAPGKQRELVAFSIDGSSTNYVDSVRGRFTASRDNAENTLYLQMNSLKPEDTAVYYCYAQGNTWAAGVWGQGTQVTVSS

SEQ ID NO: 74 - protein, 25 aa, Lama glama [sequence omitted]

SEQ ID NO: 75 - protein, 8 aa, Lama glama
ESIFSINY

SEQ ID NO: 76 - protein, 17 aa, Lama glama
MAWYRQAPGKQRELVAF

SEQ ID NO: 77 - protein, 7 aa, Lama glama
SIDGSST

SEQ ID NO: 78 - protein, 38 aa, Lama glama
NYVDSVRGRFTASRDNAENTLYLQMNSLKPEDTAVYYC

SEQ ID NO: 79 - protein, 11 aa, Lama glama
YAQGNTWAAGV

SEQ ID NO: 80 - protein, 11 aa, Lama glama
WGQGTQVTVSS

SEQ ID NO: 81 - protein, 123 aa, Lama glama
EVQLVESGGGLVQAGDSLRLSCVVSGLTFSRYGMGWFRQATGKEREFVGGISVGSSGTMYPNSVKGRFTISRDNAKSTVYLQMNSLKPEDTAVYFCAAIDQGSFVQQRDYRYWGQGTQVTVSS

SEQ ID NO: 82 - protein, 25 aa, Lama glama
EVQLVESGGGLVQAGDSLRLSCVVS

SEQ ID NO: 83 - protein, 8 aa, Lama glama
GLTFSRYG

SEQ ID NO: 84 - protein, 16 aa, Lama glama
MGWFRQATGKEREFVG

SEQ ID NO: 85 - protein, 9 aa, Lama glama
GISVGSSGT

SEQ ID NO: 86 - protein, 38 aa, Lama glama
MYPNSVKGRFTISRDNAKSTVYLQMNSLKPEDTAVYFC

SEQ ID NO: 87 - protein, 16 aa, Lama glama
AAIDQGSFVQQRDYRY

SEQ ID NO: 88 - protein, 11 aa, Lama glama
WGQGTQVTVSS

SEQ ID NO: 89 - protein, 123 aa, Lama glama
EVQLVESGGGLVQAGGSLRLSCAASGRAFGGPYMAWFRQTPGKGREFVAAISPSSVYTFYQDSVKGRFTISRDNTKNTAYLQMNSLKPEDTAVYYCAAEAAGEVRLETSYKYWGQGTQVTVSS

SEQ ID NO: 90 - protein, 25 aa, Lama glama
EVQLVESGGGLVQAGGSLRLSCAAS

SEQ ID NO: 91 - protein, 8 aa, Lama glama
GRAFGGPY

SEQ ID NO: 92 - protein, 17 aa, Lama glama
MAWFRQTPGKGREFVAA

SEQ ID NO: 93 - protein, 8 aa, Lama glama
ISPSSVYT

SEQ ID NO: 94 - protein, 38 aa, Lama glama
FYQDSVKGRFTISRDNTKNTAYLQMNSLKPEDTAVYYC

SEQ ID NO: 95 - protein, 16 aa, Lama glama
AAEAAGEVRLETSYKY

SEQ ID NO: 96 - protein, 11 aa, Lama glama
WGQGTQVTVSS

SEQ ID NO: 97 - protein, 122 aa, Lama glama
EVQLVESGGGLVQPGGSLRLSCAASGLTFVNYAMGWFRQAPGKERELVAGIASSGRIYYADSVAGRFTISRDNARNTVNLQMNSMKPEDTAVYYCAGRRSFSSTSAADYNYWGQGTQVTVSS

SEQ ID NO: 98 - protein, 25 aa, Lama glama [sequence omitted]

SEQ ID NO: 99 - protein, 8 aa, Lama glama
GLTFVNYA

SEQ ID NO: 100 - protein, 17 aa, Lama glama
MGWFRQAPGKERELVAG

SEQ ID NO: 101 - protein, 7 aa, Lama glama
IASSGRI

SEQ ID NO: 102 - protein, 38 aa, Lama glama
YYADSVAGRFTISRDNARNTVNLQMNSMKPEDTAVYYC

SEQ ID NO: 103 - protein, 16 aa, Lama glama
AGRRSFSSTSAADYNY

SEQ ID NO: 104 - protein, 11 aa, Lama glama
WGQGTQVTVSS

SEQ ID NO: 105 - protein, 115 aa, Lama glama
EVQLVESGGGLLQAGGSLTLSCAASGRTFNTMGWFRQASWKEREFVASIAWVGGSVFKSDSTKGRFTVSGDNAKNTVRLQMNSLKPEDTAVYYCAARSGGTFDVWGQGTQVTVSS

SEQ ID NO: 106 - protein, 25 aa, Lama glama
EVQLVESGGGLLQAGGSLTLSCAAS

SEQ ID NO: 107 - protein, 6 aa, Lama glama
GRTFNT

SEQ ID NO: 108 - protein, 17 aa, Lama glama
MGWFRQASWKEREFVAS

SEQ ID NO: 109 - protein, 8 aa, Lama glama
IAWVGGSV

SEQ ID NO: 110 - protein, 38 aa, Lama glama
FKSDSTKGRFTVSGDNAKNTVRLQMNSLKPEDTAVYYC

SEQ ID NO: 111 - protein, 10 aa, Lama glama
AARSGGTFDV

SEQ ID NO: 112 - protein, 11 aa, Lama glama
WGQGTQVTVSS

SEQ ID NO: 113 - protein, 125 aa, Lama glama
EVQLVESGGGLVQAGGSLRLSCVISGRTSPTYPMGWFRQSPGNEREFVASINWSGGWRNYADSVKDRFTISRDDAKNTVYLQMNSLKPEDTAVYYCARGQYSSGTPVYAHEYAYWGQGTQVTVSS

SEQ ID NO: 114 - protein, 25 aa, Lama glama
EVQLVESGGGLVQAGGSLRLSCVIS

SEQ ID NO: 115 - protein, 8 aa, Lama glama
GRTSPTYP

SEQ ID NO: 116 - protein, 17 aa, Lama glama
MGWFRQSPGNEREFVAS

SEQ ID NO: 117 - protein, 8 aa, Lama glama
INWSGGWR

SEQ ID NO: 118 - protein, 38 aa, Lama glama
NYADSVKDRFTISRDDAKNTVYLQMNSLKPEDTAVYYC

SEQ ID NO: 119 - protein, 18 aa, Lama glama
ARGQYSSGTPVYAHEYAY

SEQ ID NO: 120 - protein, 11 aa, Lama glama
WGQGTQVTVSS

SEQ ID NO: 121 - protein, 115 aa, Lama glama
EVQLVESGGGLVQPGGSLRLSCVVSGSSFSSYTMGWFRRAPGKQRELVAGVSTVGDTAAADSVKGRFTISRDNAKNTVYLQMNSLKPEDTAVYYCNTYPHAYLEWGQGTQVTVSS

SEQ ID NO: 122 - protein, 25 aa, Lama glama
EVQLVESGGGLVQPGGSLRLSCVVS

SEQ ID NO: 123 - protein, 8 aa, Lama glama
GSSFSSYT

SEQ ID NO: 124 - protein, 17 aa, Lama glama
MGWFRRAPGKQRELVAG

SEQ ID NO: 125 - protein, 7 aa, Lama glama
VSTVGDT

SEQ ID NO: 126 - protein, 38 aa, Lama glama
AAADSVKGRFTISRDNAKNTVYLQMNSLKPEDTAVYYC

SEQ ID NO: 127 - protein, 9 aa, Lama glama
NTYPHAYLE

SEQ ID NO: 128 - protein, 11 aa, Lama glama
WGQGTQVTVSS

SEQ ID NO: 129 - protein, 115 aa, Lama glama
EVQLVESGGGLVQAGGSLTLSCAASGRTFNTMGWFRQAPGKEREFVASIAWVGGSVFKSDSTKGRFTVSGDNAKNTVRLQMNSLKPEDTAVYYCAARSGGTFDVWGQGTQVTVSS

SEQ ID NO: 130 - protein, 25 aa, Lama glama
EVQLVESGGGLVQAGGSLTLSCAAS

SEQ ID NO: 131 - protein, 6 aa, Lama glama
GRTFNT

SEQ ID NO: 132 - protein, 17 aa, Lama glama
MGWFRQAPGKEREFVAS

SEQ ID NO: 133 - protein, 8 aa, Lama glama
IAWVGGSV

SEQ ID NO: 134 - protein, 38 aa, Lama glama; identical to SEQ ID NO: 110

SEQ ID NO: 135 - protein, 10 aa, Lama glama
AARSGGTFDV

SEQ ID NO: 136 - protein, 11 aa, Lama glama
WGQGTQVTVSS

SEQ ID NO: 137 - protein, 125 aa, Lama glama
EVQLVESGGELVQAGGSLRLSCAVSGRTLTSYPMGWFRQAPGKEREFVAAISWSGGDTMYADSVKGRFTISRDNSKNTVYLQMNSLKPEDTADYYCARRRYSSGISRHLVDYEYWGQGTQVTVSS

SEQ ID NO: 138 - protein, 25 aa, Lama glama
EVQLVESGGELVQAGGSLRLSCAVS

SEQ ID NO: 139 - protein, 8 aa, Lama glama
GRTLTSYP

SEQ ID NO: 140 - protein, 17 aa, Lama glama
MGWFRQAPGKEREFVAA

SEQ ID NO: 141 - protein, 8 aa, Lama glama
ISWSGGDT

SEQ ID NO: 142 - protein, 38 aa, Lama glama
MYADSVKGRFTISRDNSKNTVYLQMNSLKPEDTADYYC

SEQ ID NO: 143 - protein, 18 aa, Lama glama
ARRRYSSGISRHLVDYEY

SEQ ID NO: 144 - protein, 11 aa, Lama glama
WGQGTQVTVSS

SEQ ID NO: 145 - protein, 121 aa, Lama glama
EVQLVESGGGLVQPGGSLRLSCAASESIFSINAMGWYRQTPGKQREMVASITPGGFTIYADSVKGRFTISRDNAKNTLYLQMNNLRFEDTAVYYCNAFAGSATSYHDFGSWGQGTQVTVSS

SEQ ID NO: 146 - protein, 25 aa, Lama glama [sequence omitted]

SEQ ID NO: 147 - protein, 8 aa, Lama glama
ESIFSINA

SEQ ID NO: 148 - protein, 17 aa, Lama glama
MGWYRQTPGKQREMVAS

SEQ ID NO: 149 - protein, 7 aa, Lama glama
ITPGGFT

SEQ ID NO: 150 - protein, 38 aa, Lama glama
IYADSVKGRFTISRDNAKNTLYLQMNNLRFEDTAVYYC

SEQ ID NO: 151 - protein, 15 aa, Lama glama
NAFAGSATSYHDFGS

SEQ ID NO: 152 - protein, 11 aa, Lama glama
WGQGTQVTVSS

SEQ ID NO: 153 - protein, 122 aa, Lama glama
EVQLVESGGGLVQAGGSLRLSCAASGRSFSSSVMGWFRQTPGKEREFVAATRWTAASTHYADSVKGRFTISRDHAENAVFLQMNSLKPEDTAVYYCAAGNYLDTAQYRYNYWGQGTQVTVSS

SEQ ID NO: 154 - protein, 25 aa, Lama glama
EVQLVESGGGLVQAGGSLRLSCAAS

SEQ ID NO: 155 - protein, 8 aa, Lama glama
GRSFSSSV

SEQ ID NO: 156 - protein, 17 aa, Lama glama
MGWFRQTPGKEREFVAA

SEQ ID NO: 157 - protein, 8 aa, Lama glama
TRWTAAST

SEQ ID NO: 158 - protein, 38 aa, Lama glama
HYADSVKGRFTISRDHAENAVFLQMNSLKPEDTAVYYC

SEQ ID NO: 159 - protein, 15 aa, Lama glama
AAGNYLDTAQYRYNY

SEQ ID NO: 160 - protein, 11 aa, Lama glama
WGQGTQVTVSS

SEQ ID NO: 161 - protein, 124 aa, Lama glama
EVQLVESGGGLVQIGDSLRLSCAASGGTFNRYGMGWFRQAPGKEREFVAAIRWDGVDTNYADFVKGRFTISRYNAKNTAYLQMNSLKPEDTAVYYCAADRRGLYTKHAHRYDYWGQGTQVTVSS

SEQ ID NO: 162 - protein, 25 aa, Lama glama
EVQLVESGGGLVQIGDSLRLSCAAS

SEQ ID NO: 163 - protein, 8 aa, Lama glama
GGTFNRYG

SEQ ID NO: 164 - protein, 17 aa, Lama glama
MGWFRQAPGKEREFVAA

SEQ ID NO: 165 - protein, 8 aa, Lama glama
IRWDGVDT

SEQ ID NO: 166 - protein, 38 aa, Lama glama
NYADFVKGRFTISRYNAKNTAYLQMNSLKPEDTAVYYC

SEQ ID NO: 167 - protein, 17 aa, Lama glama
AADRRGLYTKHAHRYDY

SEQ ID NO: 168 - protein, 11 aa, Lama glama
WGQGTQVTVSS

SEQ ID NO: 169 - protein, 113 aa, Lama glama
EVQLVESGGGLVQAGGSLRLSCAASGSIVSFNGINWYRQAPGKQREWVGGITQGGNTMYADSVRGRFTISRDNTKNTMYLQMNSLKPEDTAVYYCRRPPVASWGQGTQVTVSS

SEQ ID NO: 170 - protein, 25 aa, Lama glama
EVQLVESGGGLVQAGGSLRLSCAAS

SEQ ID NO: 171 - protein, 8 aa, Lama glama
GSIVSFNG

SEQ ID NO: 172 - protein, 17 aa, Lama glama
INWYRQAPGKQREWVGG

SEQ ID NO: 173 - protein, 7 aa, Lama glama
ITQGGNT

SEQ ID NO: 174 - protein, 38 aa, Lama glama
MYADSVRGRFTISRDNTKNTMYLQMNSLKPEDTAVYYC

SEQ ID NO: 175 - protein, 7 aa, Lama glama
RRPPVAS

SEQ ID NO: 176 - protein, 11 aa, Lama glama
WGQGTQVTVSS

SEQ ID NO: 177 - protein, 122 aa, Lama glama
EVQLVESGGGLVQAGDSLRLSCTVSGRTFNTYVTGWFRQAPGKEREFVAAIHQIGSTYYRNSVKGRFTISRDGAKDTVYLQMNNLKPEDSAVYYCAAGNGGYVMSDIAYGTWGQGTQVTVSS

SEQ ID NO: 178 - protein, 25 aa, Lama glama
EVQLVESGGGLVQAGDSLRLSCTVS

SEQ ID NO: 179 - protein, 8 aa, Lama glama
GRTFNTYV

SEQ ID NO: 180 - protein, 17 aa, Lama glama
TGWFRQAPGKEREFVAA

SEQ ID NO: 181 - protein, 7 aa, Lama glama
IHQIGST

SEQ ID NO: 182 - protein, 38 aa, Lama glama
YYRNSVKGRFTISRDGAKDTVYLQMNNLKPEDSAVYYC

SEQ ID NO: 183 - protein, 16 aa, Lama glama
AAGNGGYVMSDIAYGT

SEQ ID NO: 184 - protein, 11 aa, Lama glama
WGQGTQVTVSS

SEQ ID NO: 185 - protein, 124 aa, Lama glama
EVQLVESGGGLVQAGGSLRLSCAASRGTFGTDIMGWFRQAPGKEREFVAAISWRGANTYYGYSVKGRFTISRDNAKNTMYLQMADLKPEDTADYYCGVHLNGTPYYYASGYRYWGQGTQVTVSS

SEQ ID NO: 186 - protein, 24 aa, Lama glama
EVQLVESGGGLVQAGGSLRLSCAA

SEQ ID NO: 187 - protein, 9 aa, Lama glama
SRGTFGTDI

SEQ ID NO: 188 - protein, 17 aa, Lama glama
MGWFRQAPGKEREFVAA

SEQ ID NO: 189 - protein, 8 aa, Lama glama
ISWRGANT

SEQ ID NO: 190 - protein, 38 aa, Lama glama
YYGYSVKGRFTISRDNAKNTMYLQMADLKPEDTADYYC

SEQ ID NO: 191 - protein, 17 aa, Lama glama
GVHLNGTPYYYASGYRY

SEQ ID NO: 192 - protein, 11 aa, Lama glama
WGQGTQVTVSS

SEQ ID NO: 193 - protein, 124 aa, Lama glama
EVQLVESGGGLVQAGGSLRLSCAASRGTFGTYIMGWFRQAPGKEREFVAAISWRGANTYYGYSVKGRFTISRDNAKNTMYLQMADLKPEDTADYYCGVHLNGTPYYYASGYRYWGQGTQVTVSS

SEQ ID NO: 194 - protein, 25 aa, Lama glama
EVQLVESGGGLVQAGGSLRLSCAAS

SEQ ID NO: 195 - protein, 8 aa, Lama glama
RGTFGTYI

SEQ ID NO: 196 - protein, 17 aa, Lama glama
MGWFRQAPGKEREFVAA

SEQ ID NO: 197 - protein, 8 aa, Lama glama
ISWRGANT

SEQ ID NO: 198 - protein, 38 aa, Lama glama; identical to SEQ ID NO: 190

SEQ ID NO: 199 - protein, 17 aa, Lama glama
GVHLNGTPYYYASGYRY

SEQ ID NO: 200 - protein, 11 aa, Lama glama
WGQGTQVTVSS

SEQ ID NO: 201 - protein, 118 aa, Lama glama
EVQLVESGGGTVQAGDSLRLSCTASGRTFSTYTMGWFRQAPGKERVVVAVNTWNNFTVHQPSVKGRFTMSRDNTKNSIYLQMDSLKPEDTAVYYCAASAKGTARYDYWGQGTQVTVSS

SEQ ID NO: 202 - protein, 25 aa, Lama glama
EVQLVESGGGTVQAGDSLRLSCTAS

SEQ ID NO: 203 - protein, 8 aa, Lama glama
GRTFSTYT

SEQ ID NO: 204 - protein, 17 aa, Lama glama
MGWFRQAPGKERVVVAV

SEQ ID NO: 205 - protein, 7 aa, Lama glama
NTWNNFT

SEQ ID NO: 206 - protein, 38 aa, Lama glama
VHQPSVKGRFTMSRDNTKNSIYLQMDSLKPEDTAVYYC

SEQ ID NO: 207 - protein, 12 aa, Lama glama
AASAKGTARYDY

SEQ ID NO: 208 - protein, 11 aa, Lama glama
WGQGTQVTVSS

SEQ ID NO: 209 - protein, 116 aa, Lama glama
EVQLVESGGGLVQAGGSLRLSCAASGSLRSINTMAWHRRAPGKEREWVATITGSDETIVADSVKGRFAISRDAANNTLSLEMNGLKPEDTAVYYCAAFTATLVPYWGQGTQVTVSS

SEQ ID NO: 210 - protein, 25 aa, Lama glama
EVQLVESGGGLVQAGGSLRLSCAAS

SEQ ID NO: 211 - protein, 8 aa, Lama glama
GSLRSINT

SEQ ID NO: 212 - protein, 17 aa, Lama glama
MAWHRRAPGKEREWVAT

SEQ ID NO: 213 - protein, 7 aa, Lama glama
ITGSDET

SEQ ID NO: 214 - protein, 38 aa, Lama glama
IVADSVKGRFAISRDAANNTLSLEMNGLKPEDTAVYYC

SEQ ID NO: 215 - protein, 10 aa, Lama glama
AAFTATLVPY

SEQ ID NO: 216 - protein, 11 aa, Lama glama
WGQGTQVTVSS

SEQ ID NO: 217 - protein, 115 aa, Lama glama
EVQLVESGGGLVQPGGSLRLSCAASGSLGSNNPMAWYRQAPGKERELVASISSAYRTHYADFVKGRFTISRDSPKNTVSLQMNNLKPEDTAVYYCGIFVSARNYWGKGTQVTVSS

SEQ ID NO: 218 - protein, 25 aa, Lama glama [sequence omitted]

SEQ ID NO: 219 - protein, 8 aa, Lama glama
GSLGSNNP

SEQ ID NO: 220 - protein, 17 aa, Lama glama
MAWYRQAPGKERELVAS

SEQ ID NO: 221 - protein, 7 aa, Lama glama
ISSAYRT

SEQ ID NO: 222 - protein, 38 aa, Lama glama
HYADFVKGRFTISRDSPKNTVSLQMNNLKPEDTAVYYC

SEQ ID NO: 223 - protein, 9 aa, Lama glama
GIFVSARNY

SEQ ID NO: 224 - protein, 11 aa, Lama glama
WGKGTQVTVSS

SEQ ID NO: 225 - protein, 125 aa, Lama glama
EVQLVESGGGLVQAGGSLRLSCTPSITTAGTTIMAWFRQAPGNEREFVAAIWGSKTAYGDSMKGRLTISRDNVRDNGQKTVFLQMNNLQLQDTATYYCAASSGGYVHSSTSYEIWGRGTQVTVSS

SEQ ID NO: 226 - protein, 25 aa, Lama glama
EVQLVESGGGLVQAGGSLRLSCTPS

SEQ ID NO: 227 - protein, 8 aa, Lama glama
ITTAGTTI

SEQ ID NO: 228 - protein, 17 aa, Lama glama
MAWFRQAPGNEREFVAA

SEQ ID NO: 229 - protein, 10 aa, Lama glama
IWGSKTAYGD

SEQ ID NO: 230 - protein, 38 aa, Lama glama
SMKGRLTISRDNVRDNGQKTVFLQMNNLQLQDTATYYC

SEQ ID NO: 231 - protein, 16 aa, Lama glama
AASSGGYVHSSTSYEI

SEQ ID NO: 232 - protein, 11 aa, Lama glama
WGRGTQVTVSS

SEQ ID NO: 233 - protein, 115 aa, Lama glama
EVQLVESGGGLVQAGGSLRLSCAASGIIFSANTVGWYRQVPGKERDVVASITSGDSTYYGDSVRDRFTISRDNAKNTVYLQMNSLKPDDTAIYYCRARTTDGSYWGQGTQVTVSS

SEQ ID NO: 234 - protein, 26 aa, Lama glama
EVQLVESGGGLVQAGGSLRLSCAASG

SEQ ID NO: 235 - protein, 8 aa, Lama glama
IIFSANTV

SEQ ID NO: 236 - protein, 15 aa, Lama glama
GWYRQVPGKERDVVA

SEQ ID NO: 237 - protein, 11 aa, Lama glama
SITSGDSTYYG

SEQ ID NO: 238 - protein, 35 aa, Lama glama
DSVRDRFTISRDNAKNTVYLQMNSLKPDDTAIYYC

SEQ ID NO: 239 - protein, 9 aa, Lama glama
RARTTDGSY

SEQ ID NO: 240 - protein, 11 aa, Lama glama
WGQGTQVTVSS

SEQ ID NO: 241 - protein, 114 aa, Lama glama
EVQLVESGGGLVQAGGSLRLSCAASGLTFSRYTMSWYRQAPGKEREVVAAISSGDSTYHEDSVKGRFIISRDNAKNTVYLQMNSLKTEDTAVYYCRANGPGTYWGQGTQVTVSS

SEQ ID NO: 242 - protein, 26 aa, Lama glama
EVQLVESGGGLVQAGGSLRLSCAASG

SEQ ID NO: 243 - protein, 7 aa, Lama glama
LTFSRYT

SEQ ID NO: 244 - protein, 16 aa, Lama glama
MSWYRQAPGKEREVVA

SEQ ID NO: 245 - protein, 11 aa, Lama glama
AISSGDSTYHE

SEQ ID NO: 246 - protein, 35 aa, Lama glama
DSVKGRFIISRDNAKNTVYLQMNSLKTEDTAVYYC

SEQ ID NO: 247 - protein, 8 aa, Lama glama
RANGPGTY

SEQ ID NO: 248 - protein, 11 aa, Lama glama
WGQGTQVTVSS

SEQ ID NO: 249 - protein, 109 aa, Lama glama
EVQLVESGGGLVQAGGSLRLSCAASRSISPMGWYRQAPGKQRELVAIMPSSGPPIYADSVQGRFTISRDNAKNTVYLQMNSLKPEDTAVYYCNVGGGYWGQGTQVTVSS

SEQ ID NO: 250 - protein, 25 aa, Lama glama
EVQLVESGGGLVQAGGSLRLSCAAS

SEQ ID NO: 251 - protein, 5 aa, Lama glama
RSISP

SEQ ID NO: 252 - protein, 16 aa, Lama glama
MGWYRQAPGKQRELVA

SEQ ID NO: 253 - protein, 11 aa, Lama glama
IMPSSGPPIYA

SEQ ID NO: 254 - protein, 35 aa, Lama glama
DSVQGRFTISRDNAKNTVYLQMNSLKPEDTAVYYC

SEQ ID NO: 255 - protein, 6 aa, Lama glama
NVGGGY

SEQ ID NO: 256 - protein, 11 aa, Lama glama
WGQGTQVTVSS

SEQ ID NO: 257 - protein, 123 aa, Lama glama
EVQLVESGGGLVPAGGSLRLSCAASGRTFSNYAMGWFRQAPGKERKFVATISWSGGVTYYADSVKGRFTISRDNAKNTVYLLMNSLKPEDTAVYYCAAKRDSSSYDHRRYDYWGQGTQVTVSS

SEQ ID NO: 258 - protein, 26 aa, Lama glama
EVQLVESGGGLVPAGGSLRLSCAASG

SEQ ID NO: 259 - protein, 7 aa, Lama glama
RTFSNYA

SEQ ID NO: 260 - protein, 16 aa, Lama glama
MGWFRQAPGKERKFVA

SEQ ID NO: 261 - protein, 11 aa, Lama glama
TISWSGGVTYY

SEQ ID NO: 262 - protein, 36 aa, Lama glama
ADSVKGRFTISRDNAKNTVYLLMNSLKPEDTAVYYC

SEQ ID NO: 263 - protein, 16 aa, Lama glama
AAKRDSSSYDHRRYDY

SEQ ID NO: 264 - protein, 11 aa, Lama glama
WGQGTQVTVSS

SEQ ID NO: 265 - protein, 112 aa, Lama glama
EVQLVESGGGLVQAGGSLRLSCSASGSIFSINYMAWYRQEPGKEREVVASMSWRGDSTYLADSVQGRFTISRNNAKNTMYLQMNSLKPEDTALYYCKANNYWGQGTQVTVSS

SEQ ID NO: 266 - protein, 26 aa, Lama glama
EVQLVESGGGLVQAGGSLRLSCSASG

SEQ ID NO: 267 - protein, 7 aa, Lama glama
SIFSINY

SEQ ID NO: 268 - protein, 16 aa, Lama glama
MAWYRQEPGKEREVVA

SEQ ID NO: 269 - protein, 11 aa, Lama glama
SMSWRGDSTYL

SEQ ID NO: 270 - protein, 36 aa, Lama glama
ADSVQGRFTISRNNAKNTMYLQMNSLKPEDTALYYC

SEQ ID NO: 271 - protein, 5 aa, Lama glama
KANNY

SEQ ID NO: 272 - protein, 11 aa, Lama glama
WGQGTQVTVSS

SEQ ID NO: 273 - protein, 124 aa, Lama glama
EVQLVESGGRLVQPGDSLRLSCAASGRTFSDNAMGWFRQAPGKERRFVAGISWAGGSTYYSDSVKGRFTISRDNAKNTVYLQMNSLKPEDTAVYYCAAGLRAWVQRMPKDYNYWGQGTQVTVSS

SEQ ID NO: 274 - protein, 26 aa, Lama glama
EVQLVESGGRLVQPGDSLRLSCAASG

SEQ ID NO: 275 - protein, 7 aa, Lama glama
RTFSDNA

SEQ ID NO: 276 - protein, 16 aa, Lama glama
MGWFRQAPGKERRFVA

SEQ ID NO: 277 - protein, 12 aa, Lama glama
GISWAGGSTYYS

SEQ ID NO: 278 - protein, 35 aa, Lama glama
DSVKGRFTISRDNAKNTVYLQMNSLKPEDTAVYYC

SEQ ID NO: 279 - protein, 17 aa, Lama glama
AAGLRAWVQRMPKDYNY

SEQ ID NO: 280 - protein, 11 aa, Lama glama
WGQGTQVTVSS

SEQ ID NO: 281 - protein, 119 aa, Lama glama
EVQLVESGGGLVQAGGSLRLSCAASGRAFSISSMSWFRQAPGKERVVVASIAWSGDSTYYADSVQGRFTISKDNAKNTLSLQMNSLKPEDTAVYYCSAYTQVSVNNRYWGQGTQVTVSS

SEQ ID NO: 282 - protein, 26 aa, Lama glama
EVQLVESGGGLVQAGGSLRLSCAASG

SEQ ID NO: 283 - protein, 7 aa, Lama glama
RAFSISS

SEQ ID NO: 284 - protein, 16 aa, Lama glama
MSWFRQAPGKERVVVA

SEQ ID NO: 285 - protein, 12 aa, Lama glama
SIAWSGDSTYYA

SEQ ID NO: 286 - protein, 35 aa, Lama glama
DSVQGRFTISKDNAKNTLSLQMNSLKPEDTAVYYC

SEQ ID NO: 287 - protein, 12 aa, Lama glama
SAYTQVSVNNRY

SEQ ID NO: 288 - protein, 11 aa, Lama glama
WGQGTQVTVSS

SEQ ID NO: 289 - protein, 114 aa, Lama glama
EVQLVESGGGLVQAGGSLRLSCAASGIIFGANTVGWYRQVPGKERDVVASITSGDSTYYGDSVRGRFTISRDNAKNTMYLQMNSLKPEDTAIYYCRARTTDGSYWGQGTQVTVS

SEQ ID NO: 290 - protein, 25 aa, Lama glama
EVQLVESGGGLVQAGGSLRLSCAAS

SEQ ID NO: 291 - protein, 8 aa, Lama glama
GIIFGANT

SEQ ID NO: 292 - protein, 17 aa, Lama glama
VGWYRQVPGKERDVVAS

SEQ ID NO: 293 - protein, 7 aa, Lama glama
ITSGDST

SEQ ID NO: 294 - protein, 38 aa, Lama glama
YYGDSVRGRFTISRDNAKNTMYLQMNSLKPEDTAIYYC

SEQ ID NO: 295 - protein, 9 aa, Lama glama
RARTTDGSY

SEQ ID NO: 296 - protein, 10 aa, Lama glama
WGQGTQVTVS

SEQ ID NO: 297 - protein, 114 aa, Lama glama
EVQLVESGGGLVQAGGSLRLSCAASGLTFSSYTMAWYRQAPGKEREVVAAISSGDSIYHEGSVQGRFIISRDNAKNTVYLQMNSLKAEDTAVYYCRANGPGTYWGQGTQVTVSS

SEQ ID NO: 298 - protein, 25 aa, Lama glama
EVQLVESGGGLVQAGGSLRLSCAAS

SEQ ID NO: 299 - protein, 8 aa, Lama glama
GLTFSSYT

SEQ ID NO: 300 - protein, 17 aa, Lama glama
MAWYRQAPGKEREVVAA

SEQ ID NO: 301 - protein, 7 aa, Lama glama
ISSGDSI

SEQ ID NO: 302 - protein, 38 aa, Lama glama
YHEGSVQGRFIISRDNAKNTVYLQMNSLKAEDTAVYYC

SEQ ID NO: 303 - protein, 8 aa, Lama glama
RANGPGTY

SEQ ID NO: 304 - protein, 11 aa, Lama glama
WGQGTQVTVSS

SEQ ID NO: 305 - protein, 114 aa, Lama glama
EVQLVESGGGLVQAGGSLRLSCAASGLTFSSYTMAWYRQAPGKEREVVAAISSGDSIYHEDSVQGRFIISRDNAKNTVYLQMNSLKAEDTAVYYCRANGPGTYWGQGTQVTVSS

SEQ ID NO: 306 - protein, 25 aa, Lama glama
EVQLVESGGGLVQAGGSLRLSCAAS

SEQ ID NO: 307 - protein, 8 aa, Lama glama
GLTFSSYT

SEQ ID NO: 308 - protein, 17 aa, Lama glama
MAWYRQAPGKEREVVAA

SEQ ID NO: 309 - protein, 7 aa, Lama glama
ISSGDSI

SEQ ID NO: 310 - protein, 38 aa, Lama glama
YHEDSVQGRFIISRDNAKNTVYLQMNSLKAEDTAVYYC

SEQ ID NO: 311 - protein, 8 aa, Lama glama
RANGPGTY

SEQ ID NO: 312 - protein, 11 aa, Lama glama
WGQGTQVTVSS

SEQ ID NO: 313 - protein, 112 aa, Lama glama
EVQLVESGGGLVQAGGSLRLSCAASGSIFRLNYMAWYRQAPGKEREVVASMSRRSDSTYLADAVQGRFTISMNNAGNTMYLQMNSLKPEDTALYYCKANDYWGQGTQVTVSS

SEQ ID NO: 314 - protein, 25 aa, Lama glama
EVQLVESGGGLVQAGGSLRLSCAAS

SEQ ID NO: 315 - protein, 8 aa, Lama glama
GSIFRLNY

SEQ ID NO: 316 - protein, 16 aa, Lama glama
MAWYRQAPGKEREVVA

SEQ ID NO: 317 - protein, 9 aa, Lama glama
SMSRRSDST

SEQ ID NO: 318 - protein, 38 aa, Lama glama
YLADAVQGRFTISMNNAGNTMYLQMNSLKPEDTALYYC

SEQ ID NO: 319 - protein, 4 aa, Lama glama
KAND

SEQ ID NO: 320 - protein, 12 aa, Lama glama
YWGQGTQVTVSS

SEQ ID NO: 321 - protein, 112 aa, Lama glama; identical to SEQ ID NO: 265

SEQ ID NO: 322 - protein, 25 aa, Lama glama
EVQLVESGGGLVQAGGSLRLSCSAS

SEQ ID NO: 323 - protein, 8 aa, Lama glama
GSIFSINY

SEQ ID NO: 324 - protein, 16 aa, Lama glama
MAWYRQEPGKEREVVA

SEQ ID NO: 325 - protein, 9 aa, Lama glama
SMSWRGDST

SEQ ID NO: 326 - protein, 38 aa, Lama glama
YLADSVQGRFTISRNNAKNTMYLQMNSLKPEDTALYYC

SEQ ID NO: 327 - protein, 5 aa, Lama glama
KANNY

SEQ ID NO: 328 - protein, 11 aa, Lama glama
WGQGTQVTVSS

SEQ ID NO: 329 - protein, 109 aa, Lama glama
EVQLVESGGGLVQAGGSLRLSCAASRSISPMGWYRQAPGKQRELVAIMPSSGTPIYADSVQGRFTISRDNAKNTVYLQMNSLKPEDTAVYYCNVGGGYWGQGTQVTVSS

SEQ ID NO: 330 - protein, 25 aa, Lama glama
EVQLVESGGGLVQAGGSLRLSCAAS

SEQ ID NO: 331 - protein, 5 aa, Lama glama
RSISP

SEQ ID NO: 332 - protein, 16 aa, Lama glama
MGWYRQAPGKQRELVA

SEQ ID NO: 333 - protein, 9 aa, Lama glama
IMPSSGTPI

SEQ ID NO: 334 - protein, 37 aa, Lama glama
YADSVQGRFTISRDNAKNTVYLQMNSLKPEDTAVYYC

SEQ ID NO: 335 - protein, 5 aa, Lama glama
NVGGG

SEQ ID NO: 336 - protein, 12 aa, Lama glama
YWGQGTQVTVSS

SEQ ID NO: 337 - protein, 115 aa, Lama glama
EVQLVESGGGLVQAGGSLRLSCAASGIIFGANTVGWYRQVPGKERDVVASITSVDSTYYGDSVRGRFTISRDNAKNTVYLQMNSLKPEDTAIYYCRARTTDGSYWGQGTQVTVSS

SEQ ID NO: 338 - protein, 25 aa, Lama glama
EVQLVESGGGLVQAGGSLRLSCAAS

SEQ ID NO: 339 - protein, 8 aa, Lama glama
GIIFGANT

SEQ ID NO: 340 - protein, 16 aa, Lama glama
VGWYRQVPGKERDVVA

SEQ ID NO: 341 - protein, 8 aa, Lama glama
SITSVDST

SEQ ID NO: 342 - protein, 38 aa, Lama glama
YYGDSVRGRFTISRDNAKNTVYLQMNSLKPEDTAIYYC

SEQ ID NO: 343 - protein, 8 aa, Lama glama
RARTTDGS

SEQ ID NO: 344 - protein, 12 aa, Lama glama
YWGQGTQVTVSS

SEQ ID NO: 345 - protein, 112 aa, Lama glama
EVQLVESGGGLVQAGGSLRLSCAASGSIFSINYMAWYRQAPGKEREVVASMSWRRDSTYLADSVQGRFTISRNNAKNTMYLQMNSLKPEDTALYYCKANDYWGQGTQVTVSS

SEQ ID NO: 346 - protein, 25 aa, Lama glama
EVQLVESGGGLVQAGGSLRLSCAAS

SEQ ID NO: 347 - protein, 8 aa, Lama glama
GSIFSINY

SEQ ID NO: 348 - protein, 16 aa, Lama glama
MAWYRQAPGKEREVVA

SEQ ID NO: 349 - protein, 9 aa, Lama glama
SMSWRRDST

SEQ ID NO: 350 - protein, 37 aa, Lama glama
YLADSVQGRFTISRNNAKNTMYLQMNSLKPEDTALYY

SEQ ID NO: 351 - protein, 5 aa, Lama glama
CKAND

SEQ ID NO: 352 - protein, 12 aa, Lama glama
YWGQGTQVTVSS

SEQ ID NO: 353 - protein, 112 aa, Lama glama
EVQLVESGGGLVQAGGSLRLSCVASGSIFSINYMAWYRQTPGKEREVVASMSRRSDSTYLADAVQGRFTISRNNAGNTMYLQMNSLKPEDTALYYCKANDYWGQGTQVTVSS

SEQ ID NO: 354 - protein, 25 aa, Lama glama
EVQLVESGGGLVQAGGSLRLSCVAS

SEQ ID NO: 355 - protein, 8 aa, Lama glama
GSIFSINY

SEQ ID NO: 356 - protein, 16 aa, Lama glama
MAWYRQTPGKEREVVA

SEQ ID NO: 357 - protein, 9 aa, Lama glama
SMSRRSDST

SEQ ID NO: 358 - protein, 37 aa, Lama glama
YLADAVQGRFTISRNNAGNTMYLQMNSLKPEDTALYY

SEQ ID NO: 359 - protein, 5 aa, Lama glama
CKAND

SEQ ID NO: 360 - protein, 12 aa, Lama glama
YWGQGTQVTVSS

SEQ ID NO: 361 - protein, 119 aa, Lama glama; identical to SEQ ID NO: 281

SEQ ID NO: 362 - protein, 26 aa, Lama glama
EVQLVESGGGLVQAGGSLRLSCAASG

SEQ ID NO: 363 - protein, 7 aa, Lama glama
RAFSISS

SEQ ID NO: 364 - protein, 16 aa, Lama glama
MSWFRQAPGKERVVVA

SEQ ID NO: 365 - protein, 12 aa, Lama glama
SIAWSGDSTYYA

SEQ ID NO: 366 - protein, 35 aa, Lama glama; identical to SEQ ID NO: 286

SEQ ID NO: 367 - protein, 12 aa, Lama glama
SAYTQVSVNNRY

SEQ ID NO: 368 - protein, 11 aa, Lama glama
WGQGTQVTVSS

SEQ ID NO: 369 - protein, 15 aa, synthetic construct
  REGION 1..15: note = Gly-Gly-Gly-Gly-Ser linker
GGGGSGGGGSGGGGS

SEQ ID NO: 370 - protein, 6 aa, synthetic construct
  REGION 1..6: note = hexahistidine-tag
HHHHHH

SEQ ID NO: 371 - protein, 4 aa, synthetic construct
  REGION 1..4: note = EPEA-tag
EPEA